European Patent Application EP 4 643 952 A2, published November 5, 2025. Title: TARGETING CHROMATIN REGULATORS INHIBITS LEUKEMOGENIC GENE EXPRESSION IN NPM1 MUTANT LEUKEMIA. Applicant: MEMORIAL SLOAN KETTERING CANCER CENTER. The sequence listing filed with the application follows.

SEQUENCE LISTING (65 sequences)

SEQ ID NO: 1 - DNA, 23 bp, synthetic construct
  misc_feature 1..23: note = Description of Artificial Sequence: Synthetic oligonucleotide
  source 1..23: mol_type = other DNA
cgccccgcggcaacgcgtcccgg

SEQ ID NO: 2 - DNA, 23 bp, synthetic construct
  misc_feature 1..23: note = Description of Artificial Sequence: Synthetic oligonucleotide
  source 1..23: mol_type = other DNA
gggccgccaccgccgaccggggg

SEQ ID NO: 3 - DNA, 23 bp, synthetic construct
  misc_feature 1..23: note = Description of Artificial Sequence: Synthetic oligonucleotide
  source 1..23: mol_type = other DNA
cgaagacgaggcggacgacgagg

SEQ ID NO: 4 - DNA, 23 bp, synthetic construct
  misc_feature 1..23: note = Description of Artificial Sequence: Synthetic oligonucleotide
  source 1..23: mol_type = other DNA
tgacgaagacgaagacgaggcgg

SEQ ID NO: 5 - DNA, 23 bp, synthetic construct
  misc_feature 1..23: note = Description of Artificial Sequence: Synthetic oligonucleotide
  source 1..23: mol_type = other DNA
tgcagcgccgcgtcgaagcccgg

SEQ ID NO: 6 - DNA, 23 bp, synthetic construct
  misc_feature 1..23: note = Description of Artificial Sequence: Synthetic oligonucleotide
  source 1..23: mol_type = other DNA
gcaccaacctgcgccggttccgg

SEQ ID NO: 7 - DNA, 23 bp, synthetic construct
  misc_feature 1..23: note = Description of Artificial Sequence: Synthetic oligonucleotide
  source 1..23: mol_type = other DNA
ctgcaggtctcggccgccatcgg

SEQ ID NO: 8 - DNA, 23 bp, synthetic construct
  misc_feature 1..23: note = Description of Artificial Sequence: Synthetic oligonucleotide
  source 1..23: mol_type = other DNA
ggtgggcccgggcttcgacgcgg

SEQ ID NO: 9 - DNA, 23 bp, synthetic construct
  misc_feature 1..23: note = Description of Artificial Sequence: Synthetic oligonucleotide
  source 1..23: mol_type = other DNA
gacgtcgatcgaggcggtgtggg

SEQ ID NO: 10 - DNA, 23 bp, synthetic construct
  misc_feature 1..23: note = Description of Artificial Sequence: Synthetic oligonucleotide
  source 1..23: mol_type = other DNA
tatattgcgaccaccaaacttgg

SEQ ID NO: 11 - DNA, 23 bp, synthetic construct
  misc_feature 1..23: note = Description of Artificial Sequence: Synthetic oligonucleotide
  source 1..23: mol_type = other DNA
tgcttagataagcccaagtttgg

SEQ ID NO: 12 - DNA, 23 bp, synthetic construct
  misc_feature 1..23: note = Description of Artificial Sequence: Synthetic oligonucleotide
  source 1..23: mol_type = other DNA
gtacaaacaccacagtcctcagg

SEQ ID NO: 13 - DNA, 23 bp, synthetic construct
  misc_feature 1..23: note = Description of Artificial Sequence: Synthetic oligonucleotide
  source 1..23: mol_type = other DNA
agaggagaacgagcgccctctgg

SEQ ID NO: 14 - DNA, 23 bp, synthetic construct
  misc_feature 1..23: note = Description of Artificial Sequence: Synthetic oligonucleotide
  source 1..23: mol_type = other DNA
tgcaaattctgtcacgtttgtgg

SEQ ID NO: 15 - DNA, 23 bp, synthetic construct
  misc_feature 1..23: note = Description of Artificial Sequence: Synthetic oligonucleotide
  source 1..23: mol_type = other DNA
actcagggtgatagctgtttcgg

SEQ ID NO: 16 - DNA, 23 bp, synthetic construct
  misc_feature 1..23: note = Description of Artificial Sequence: Synthetic oligonucleotide
  source 1..23: mol_type = other DNA
tgtgagacagcaacccacggtgg

SEQ ID NO: 17 - DNA, 23 bp, synthetic construct
  misc_feature 1..23: note = Description of Artificial Sequence: Synthetic oligonucleotide
  source 1..23: mol_type = other DNA
acacatgaagtgatagttgctgg

SEQ ID NO: 18 - DNA, 23 bp, synthetic construct
  misc_feature 1..23: note = Description of Artificial Sequence: Synthetic oligonucleotide
  source 1..23: mol_type = other DNA
ccatttgctacgctaccggcagg

SEQ ID NO: 19 - DNA, 23 bp, synthetic construct
  misc_feature 1..23: note = Description of Artificial Sequence: Synthetic oligonucleotide
  source 1..23: mol_type = other DNA
gtctcgggatttaagtctggagg

SEQ ID NO: 20 - DNA, 23 bp, synthetic construct
  misc_feature 1..23: note = Description of Artificial Sequence: Synthetic oligonucleotide
  source 1..23: mol_type = other DNA
tggtggatcaggtccttcggggg

SEQ ID NO: 21 - DNA, 23 bp, synthetic construct
  misc_feature 1..23: note = Description of Artificial Sequence: Synthetic oligonucleotide
  source 1..23: mol_type = other DNA
cagcagcctttagatctagaagg

SEQ ID NO: 22 - DNA, 23 bp, synthetic construct
  misc_feature 1..23: note = Description of Artificial Sequence: Synthetic oligonucleotide
  source 1..23: mol_type = other DNA
gatggagcggatgacgttgccgg

SEQ ID NO: 23 - DNA, 23 bp, synthetic construct
  misc_feature 1..23: note = Description of Artificial Sequence: Synthetic oligonucleotide
  source 1..23: mol_type = other DNA
aaaagaccccggccatggatggg

SEQ ID NO: 24 - DNA, 23 bp, synthetic construct
  misc_feature 1..23: note = Description of Artificial Sequence: Synthetic oligonucleotide
  source 1..23: mol_type = other DNA
ggaaaagtattacgacagcaagg

SEQ ID NO: 25 - DNA, 23 bp, synthetic construct
  misc_feature 1..23: note = Description of Artificial Sequence: Synthetic oligonucleotide
  source 1..23: mol_type = other DNA
gagatggtgattgagtatgccgg

SEQ ID NO: 26 - DNA, 23 bp, synthetic construct
  misc_feature 1..23: note = Description of Artificial Sequence: Synthetic oligonucleotide
  source 1..23: mol_type = other DNA
ccccgttgccccgtccgccgcgg

SEQ ID NO: 27 - DNA, 23 bp, synthetic construct
  misc_feature 1..23: note = Description of Artificial Sequence: Synthetic oligonucleotide
  source 1..23: mol_type = other DNA
caacggggccgaaagagtgcggg

SEQ ID NO: 28 - DNA, 23 bp, synthetic construct
  misc_feature 1..23: note = Description of Artificial Sequence: Synthetic oligonucleotide
  source 1..23: mol_type = other DNA
acggccctgctccgtttgctggg

SEQ ID NO: 29 - DNA, 23 bp, synthetic construct
  misc_feature 1..23: note = Description of Artificial Sequence: Synthetic oligonucleotide
  source 1..23: mol_type = other DNA
cgtttgctggggctccgccgggg

SEQ ID NO: 30 - DNA, 23 bp, synthetic construct
  misc_feature 1..23: note = Description of Artificial Sequence: Synthetic oligonucleotide
  source 1..23: mol_type = other DNA
gagccccagcaaacggagcaggg

SEQ ID NO: 31 - DNA, 23 bp, synthetic construct
  misc_feature 1..23: note = Description of Artificial Sequence: Synthetic oligonucleotide
  source 1..23: mol_type = other DNA
ggccgtgtcctccccgggctcgg

SEQ ID NO: 32 - DNA, 23 bp, synthetic construct
  misc_feature 1..23: note = Description of Artificial Sequence: Synthetic oligonucleotide
  source 1..23: mol_type = other DNA
aagatgcgcatggctcgatgtgg

SEQ ID NO: 33 - DNA, 23 bp, synthetic construct
  misc_feature 1..23: note = Description of Artificial Sequence: Synthetic oligonucleotide
  source 1..23: mol_type = other DNA
tcggggctgcctacgtgtgcagg

SEQ ID NO: 34 - DNA, 23 bp, synthetic construct
  misc_feature 1..23: note = Description of Artificial Sequence: Synthetic oligonucleotide
  source 1..23: mol_type = other DNA
ggtgttagggcccccaaacttgg

SEQ ID NO: 35 - DNA, 23 bp, synthetic construct
  misc_feature 1..23: note = Description of Artificial Sequence: Synthetic oligonucleotide
  source 1..23: mol_type = other DNA
cagctcgtggagtcctttgctgg

SEQ ID NO: 36 - DNA, 23 bp, synthetic construct
  misc_feature 1..23: note = Description of Artificial Sequence: Synthetic oligonucleotide
  source 1..23: mol_type = other DNA
agcaccaggtgtcgtgatgctgg

SEQ ID NO: 37 - DNA, 23 bp, synthetic construct
  misc_feature 1..23: note = Description of Artificial Sequence: Synthetic oligonucleotide
  source 1..23: mol_type = other DNA
ccacgcgcaaacggcgccactgg

SEQ ID NO: 38 - DNA, 23 bp, synthetic construct
  misc_feature 1..23: note = Description of Artificial Sequence: Synthetic oligonucleotide
  source 1..23: mol_type = other DNA
tgcataccacccggcctgtctgg

SEQ ID NO: 39 - DNA, 23 bp, synthetic construct
  misc_feature 1..23: note = Description of Artificial Sequence: Synthetic oligonucleotide
  source 1..23: mol_type = other DNA
agtgcgcacagtgcgatcactgg

SEQ ID NO: 40 - DNA, 23 bp, synthetic construct
  misc_feature 1..23: note = Description of Artificial Sequence: Synthetic oligonucleotide
  source 1..23: mol_type = other DNA
tcatagcagcgtgtacagatcgg

SEQ ID NO: 41 - DNA, 23 bp, synthetic construct
  misc_feature 1..23: note = Description of Artificial Sequence: Synthetic oligonucleotide
  source 1..23: mol_type = other DNA
ctggtcggcggaagtcttcgagg

SEQ ID NO: 42 - DNA, 23 bp, synthetic construct
  misc_feature 1..23: note = Description of Artificial Sequence: Synthetic oligonucleotide
  source 1..23: mol_type = other DNA
ctgaagcctggcgccacggtggg

SEQ ID NO: 43 - DNA, 23 bp, synthetic construct
  misc_feature 1..23: note = Description of Artificial Sequence: Synthetic oligonucleotide
  source 1..23: mol_type = other DNA
agctgtgagtcagcgcttcgagg

SEQ ID NO: 44 - DNA, 23 bp, synthetic construct
  misc_feature 1..23: note = Description of Artificial Sequence: Synthetic oligonucleotide
  source 1..23: mol_type = other DNA
actcacagcttgcaggccgcagg

SEQ ID NO: 45 - DNA, 23 bp, synthetic construct
  misc_feature 1..23: note = Description of Artificial Sequence: Synthetic oligonucleotide
  source 1..23: mol_type = other DNA
gatgggaagcaactgcacccagg

SEQ ID NO: 46 - DNA, 23 bp, synthetic construct
  misc_feature 1..23: note = Description of Artificial Sequence: Synthetic oligonucleotide
  source 1..23: mol_type = other DNA
cagcagtgggcccaccaccttgg

SEQ ID NO: 47 - DNA, 23 bp, synthetic construct
  misc_feature 1..23: note = Description of Artificial Sequence: Synthetic oligonucleotide
  source 1..23: mol_type = other DNA
taagcgcaacatcgacgcggggg

SEQ ID NO: 48 - DNA, 23 bp, synthetic construct
  misc_feature 1..23: note = Description of Artificial Sequence: Synthetic oligonucleotide
  source 1..23: mol_type = other DNA
cgggtgctatatgttccgcatgg

SEQ ID NO: 49 - DNA, 23 bp, synthetic construct
  misc_feature 1..23: note = Description of Artificial Sequence: Synthetic oligonucleotide
  source 1..23: mol_type = other DNA
ggcggcattgccatgcatcgtgg

SEQ ID NO: 50 - DNA, 20 bp, synthetic construct
  misc_feature 1..20: note = Description of Artificial Sequence: Synthetic primer
  source 1..20: mol_type = other DNA
gggagacgggagagtacaga

SEQ ID NO: 51 - DNA, 20 bp, synthetic construct
  misc_feature 1..20: note = Description of Artificial Sequence: Synthetic primer
  source 1..20: mol_type = other DNA
cccgagctgatgagcgagtc

SEQ ID NO: 52 - DNA, 20 bp, synthetic construct
  misc_feature 1..20: note = Description of Artificial Sequence: Synthetic primer
  source 1..20: mol_type = other DNA
agagagtccccatacgcttg

SEQ ID NO: 53 - DNA, 20 bp, synthetic construct
  misc_feature 1..20: note = Description of Artificial Sequence: Synthetic primer
  source 1..20: mol_type = other DNA
gatcgtaaaaatcgccgaga

SEQ ID NO: 54 - DNA, 20 bp, synthetic construct
  misc_feature 1..20: note = Description of Artificial Sequence: Synthetic primer
  source 1..20: mol_type = other DNA
atccagctgcagagaaaagc

SEQ ID NO: 55 - DNA, 19 bp, synthetic construct
  misc_feature 1..19: note = Description of Artificial Sequence: Synthetic primer
  source 1..19: mol_type = other DNA
ggctccctaccagcagaac

SEQ ID NO: 56 - DNA, 20 bp, synthetic construct
  misc_feature 1..20: note = Description of Artificial Sequence: Synthetic primer
  source 1..20: mol_type = other DNA
aggttttgggagaacgtgtg

SEQ ID NO: 57 - DNA, 25 bp, synthetic construct
  misc_feature 1..25: note = Description of Artificial Sequence: Synthetic primer
  source 1..25: mol_type = other DNA
cgtagcacagcttctccttaatgtc

SEQ ID NO: 58 - DNA, 20 bp, synthetic construct
  misc_feature 1..20: note = Description of Artificial Sequence: Synthetic primer
  source 1..20: mol_type = other DNA
gctctacgatggggtttgtt

SEQ ID NO: 59 - DNA, 24 bp, synthetic construct
  misc_feature 1..24: note = Description of Artificial Sequence: Synthetic primer
  source 1..24: mol_type = other DNA
gccaaattatcccacaacaatgtc

SEQ ID NO: 60 - DNA, 20 bp, synthetic construct
  misc_feature 1..20: note = Description of Artificial Sequence: Synthetic primer
  source 1..20: mol_type = other DNA
attttgggagggggagattt

SEQ ID NO: 61 - DNA, 20 bp, synthetic construct
  misc_feature 1..20: note = Description of Artificial Sequence: Synthetic primer
  source 1..20: mol_type = other DNA
tgtcaactccccaaaaccat

SEQ ID NO: 62 - DNA, 20 bp, synthetic construct
  misc_feature 1..20: note = Description of Artificial Sequence: Synthetic primer
  source 1..20: mol_type = other DNA
gttaggttactggcgggttg

SEQ ID NO: 63 - DNA, 19 bp, synthetic construct
  misc_feature 1..19: note = Description of Artificial Sequence: Synthetic primer
  source 1..19: mol_type = other DNA
gaataggctctggcgttgc

SEQ ID NO: 64 - DNA, 20 bp, synthetic construct
  misc_feature 1..20: note = Description of Artificial Sequence: Synthetic primer
  source 1..20: mol_type = other DNA
cctttagcacttcgcaggag

SEQ ID NO: 65 - DNA, 18 bp, synthetic construct
  misc_feature 1..18: note = Description of Artificial Sequence: Synthetic primer
  source 1..18: mol_type = other DNA
agcgcggctacagcttca